European Patent Application EP 4 458 854 A1, published November 6, 2024. Title: GPRC5D Antibody and Application Thereof. Applicant: Shandong Simcere Biopharmaceutical Co.,Ltd. The sequence listing filed with the application follows.

SEQUENCE LISTING (243 sequences)

SEQ ID NO: 1 - protein, 118 aa, Synthetic Construct
QVQLVQSGAEVKKPGASVKVSCKASGYSFTGYTMNWVRQAPGQGLEWMGLINPYNSDTNYAQKLQGRVTMTTDTSTSTAYMELRSLRSDDTAVYYCARVALRVALDYWGQGTLVTVSS

SEQ ID NO: 2 - protein, 107 aa, Synthetic Construct
DIQMTQSPSSLSASVGDRVTITCKASQNVATHVGWYQQKPGKAPKRLIYSASYRYSGVPSRFSGSGSGTEFTLTISNLQPEDFATYYCQQYNRYPYTFGQGTKLEIK

SEQ ID NO: 3 - protein, 116 aa, Synthetic Construct
EVQLVESGGGLVQPGRSLKLSCAASGFSFSNYGMAWVRQAATKGLEWVASISTGGGNTYYRDSVKGRFIVSRDNAKNTQYLQMDSLRSEDTATYYCTRHDRGGLYWGQGVMVTVSS

SEQ ID NO: 4 - protein, 112 aa, Synthetic Construct
DIVMTQAPLSVSVTPGESASISCRSSKSLLHSNGITYVYWYFQKPGKSPQVLIYRMSNLASGVPDRFSGSGSETDFTLKISRVEAEDVGIYHCGQLLENPYTFGAGTELELK

SEQ ID NO: 5 - protein, 330 aa, Synthetic Construct
ASTKGPSVFPLAPSSKSTSGGTAALGCLVKDYFPEPVTVSWNSGALTSGVHTFPAVLQSSGLYSLSSVVTVPSSSLGTQTYICNVNHKPSNTKVDKKVEPKSCDKTHTCPPCPAPELLGGPSVFLFPPKPKDTLMISRTPEVTCVVVDVSHEDPEVKFNWYVDGVEVHNAKTKPREEQYNSTYRVVSVLTVLHQDWLNGKEYKCKVSNKALPAPIEKTISKAKGQPREPQVYTLPPSREEMTKNQVSLTCLVKGFYPSDIAVEWESNGQPENNYKTTPPVLDSDGSFFLYSKLTVDKSRWQQGNVFSCSVMHEALHNHYTQKSLSLSPGK

SEQ ID NO: 6 - protein, 107 aa, Synthetic Construct [sequence omitted]

SEQ ID NO: 7 - protein, 232 aa, Synthetic Construct
EPKSSDKTHTCPPCPAPELLGGPSVFLFPPKPKDTLMISRTPEVTCVVVDVSHEDPEVKFNWYVDGVEVHNAKTKPREEQYNSTYRVVSVLTVLHQDWLNGKEYKCKVSNKALPAPIEKTISKAKGQPREPQVYTLPPSREEMTKNQVSLTCLVKGFYPSDIAVEWESNGQPENNYKTTPPVLDSDGSFFLYSKLTVDKSRWQQGNVFSCSVMHEALHNHYTQKSLSLSPGK

SEQ ID NO: 8 - protein, 357 aa, Homo sapiens
MATTVPDGCRNGLKSKYYRLCDKAEAWGIVLETVATAGVVTSVAFMLTLPILVCKVQDSNRRKMLPTQFLFLLGVLGIFGLTFAFIIGLDGSTGPTRFFLFGILFSICFSCLLAHAVSLTKLVRGRKPLSLLVILGLAVGFSLVQDVIAIEYIVLTMNRTNVNVFSELSAPRRNEDFVLLLTYVLFLMALTFLMSSFTFCGSFTGWKRHGAHIYLTMLLSIAIWVAWITLLMLPDFDRRWDDTILSSALAANGWVFLLAYVSPEFWLLTKQRNPMDYPVEDAFCKPQLVKKSYGVENRAYSQEEITQGFEETGDTLYAPYSTHFQLQNQPPQKEFSIPRAHAWPSPYKDYEVKKEGS

SEQ ID NO: 9 - protein, 375 aa, Homo sapiens
ENASTSRGCGLDLLPQYVSLCDLDAIWGIVVEAVAGAGALITLLLMLILLVRLPFIKEKEKKSPVGLHFLFLLGTLGLFGLTFAFIIQEDETICSVRRFLWGVLFALCFSCLLSQAWRVRRLVRHGTGPAGWQLVGLALCLMLVQVIIAVEWLVLTVLRDTRPACAYEPMDFVMALIYDMVLLVVTLGLALFTLCGKFKRWKLNGAFLLITAFLSVLIWVAWMTMYLFGNVKLQQGDAWNDPTLAITLAASGWVFVIFHAIPEIHCTLLPALQENTPNYFDTSQPRMRETAFEEDVQLPRAYMENKAFSMDEHNAALRTAGFPNGSLGKRPSGSLGKRPSAPFRSNVYQPTEMAVVLNGGTIPTAPPSHTGRHLW

SEQ ID NO: 10 - protein, 418 aa, Homo sapiens
QGHVPPGCSQGLNPLYYNLCDRSGAWGIVLEAVAGAGIVTTFVLTIILVASLPFVQDTKKRSLLGTQVFFLLGTLGLFCLVFACVVKPDFSTCASRRFLFGVLFAICFSCLAAHVFALNFLARKNHGPRGWVIFTVALLLTLVEVIINTEWLIITLVRGSGEGGPQGNSSAGWAVASPCAIANMDFVMALIYVMLLLLGAFLGAWPALCGRYKRWRKHGVFVLLTTATSVAIWVVWIVMYTYGNKQHNSPTWDDPTLAIALAANAWAFVLFYVIPEVSQVTKSSPEQSYQGDMYPTRGVGYETILKEQKGQSMFVENKAFSMDEPVAAKRPVSPYSGYNGQLLTSVYQPTEMALMHKVPSEGAYDIILPRATANSQVMGSANSTLRAEDMYSAQSHQAATPPKDGKNSQVFRNPYVWD

SEQ ID NO: 11 - protein, 345 aa, Homo sapiens
MYKDCIESTGDYFLLCDAEGPWGIILESLAILGIVVTILLLLAFLFLMRKIQDCSQWNVLPTQLLFLLSVLGLFGLAFAFIIELNQQTAPVRYFLFGVLFALCFSCLLAHASNLVKLVRGCVSFSWTTILCIAIGCSLLQIIIATEYVTLIMTRGMMFVNMTPCQLNVDFVVLLVYVLFLMALTFFVSKATFCGPCENWKQHGRLIFITVLFSIIIWVVWISMLLRGNPQFQRQPQWDDPVVCIALVTNAWVFLLLYIVPELCILYRSCRQECPLQGNACPVTAYQHSFQVENQELSRARDSDGAEEDVALTSYGTPIQPQTVDPTQECFIPQAKLSPQQDAGGV

SEQ ID NO: 12 - protein, 344 aa, Cynomolgus Macaques
MYKDCIESTGDYFLPCDSEGPWGIVLESLAILGIVVTILLLLAFLFLMRKIQDCSQWNVLPTQLLFLLSVLGLFGLAFAFIIQLNQQTAPVRYFLFGVLFALCFSCLLAHASNLVKLVRGRVSFSWTTILCIAIGCSLLQVIIAIEYVTLIMTRGMMFVHMTPYQLNVDFVVLLVYVLFLMALTFFVSKATFCGPCENWKQHGRLIFITVLFSIIIWVVWISMLLRGNPQFQRQPQWDDPVVCIALVTNAWVFLLLYIVPELCILYRSCRQECPSQGHACPVTAYQRSFQVENQELSRARDSDGAEEDVALTSFGTPIQPQTVDPTQECFIPRAKLSPQQDAGV

SEQ ID NO: 13 - protein, 122 aa, Synthetic Construct
QVQLKESGPGLVAPSQSLSITCTVSGFSLTNYGVSWVRQPPGKGLEWLGVIWGDGSTNYHSALISRLSIRKDNSKSQVFLKLNSLQTDDTATYYCAKPASYYGRRTYAMDFWGHGTSVTVSS

SEQ ID NO: 14 - protein, 107 aa, Synthetic Construct
QIVLSQSPAILSASPGEKVTMTCRASSSVSYMHWYQQKPGSSPKPWIYATSHLASGVPARFSGSGSGTSYSLTISRVEAEDAATYYCQQWSSNPPMTFGGGTKLEIK

SEQ ID NO: 15 - protein, 121 aa, Synthetic Construct
QVQLQQPGAELVKPGASVKMSCKASGYTFSSYWITWVKQRPGQGLDWIGDFYPRNGDTNYNKKFKNKATLTVDTSSSTAYMQLSSLTSEDSAVYYCARSRAYYGRRGFDYWGQGTTLTVSS

SEQ ID NO: 16 - protein, 106 aa, Synthetic Construct
QIVLTQSPAIMSASPGEKVTMTCSAGSSVSYMYWYQQKPGSSPRVLIYDTSNLASGVPVRFSGSGSGTSYSLIISRMEAEDAATYYCQQWSNYPLTFGAGTKLELK

SEQ ID NO: 17 - protein, 118 aa, Synthetic Construct
QAYLQQSGAELVRPGASVKMSCKASGYTFTSYNMNWVKQTPRQGLEWIGAIYPGNGDTSYNQKFKGKATLTVDKSSSTAYMQLSSLTSEDSAVYFCARVRLRYAMDYWGQGTSVTVSS

SEQ ID NO: 18 - protein, 107 aa, Synthetic Construct
DIVMTQSQKFMSTTVGDRVTITCKASQNVGTAVAWYQQKPGQSPKLLISSASNRYTGVPERFTGSGSGTDFTLTIRNMQSEDLADYFCQQYSSYPWTFGGGTELEIK

SEQ ID NO: 19 - protein, 122 aa, Synthetic Construct
EVQLVESGGGLVKPGGSLKLSCAASRFTFSRYAMSWVRQTPEKRLEWVATISDGGSYTYYPDNVKGRFTISRDNAKNNLYLQMSHLKSEDTAIYYCARDRYYYGKGGYFDVWGTGTTVTVSS

SEQ ID NO: 20 - protein, 107 aa, Synthetic Construct
DIQMTQSPASLSVSVGETVTITCRASENIYRNLAWYQQKQGKSPQLLVYAATNLADGVPSRFSGSGSGTQYSLKINSLQSEDFGSYYCQHFWGTPRTFGGGTKLEIK

SEQ ID NO: 21 - protein, 121 aa, Synthetic Construct
QVQLQQSGAELARPGASVMLSCKASGYTFTSYGISWVKQRTGQGLEWIGEIYPRSGNTYYNEKFKGKATLTADKSSSTAYMELRSLTSEDSAVYFCARGRAYGRNYPMDYWGQGTSVTVSS

SEQ ID NO: 22 - protein, 107 aa, Synthetic Construct
DILLTQSPAILSVSVGERVSFSCRASQSIGTSIHWYQQRTNGSPRLLIKYASESISGIPSRFSGSGSGTDFTLSINSVESEDIADYYCQQSNSWPYTFGGGTKLEIK

SEQ ID NO: 23 - protein, 120 aa, Synthetic Construct
QVQLKQSGPGLVQPSQSLSITCTVSGFSLTSYGVNWIRQSPGKGLEWLGVIWSGGNTDYNAAFRSRLSISKDNSKSQVFFKMNSLQADDTAIYYCARGQLGRPYWYFDVWGTGTSVTVSS

SEQ ID NO: 24 - protein, 107 aa, Synthetic Construct
DIVMTQSHKFMSTSVGDRVSITCKASQDVRTAVAWYQQKPGQSPKLLIYWASTRHTGVPDRFTGSRSGTDYTLTISSVQAEDLALYYCQQHYSTPLTFGAGTKLELK

SEQ ID NO: 25 - protein, 113 aa, Synthetic Construct
QVQLQQSGAEVVRPGTSVKVSCKASGYAFTNYLIEWLKQRPGQGLEWIGMINPGRGNTNYNEKFKGKATLTADKASSTAYMQISSLTSEDSAVYFCARNWDVWGQGTTLTVSS

SEQ ID NO: 26 - protein, 112 aa, Synthetic Construct
DVVMTQTPLSLPVSLGDQASISCRSSQSLVYSNGNTYLHWYLQKPGQSPKLLIYKVSNRFSGVPDRFSGSGSGTDFTLKISRVEAEDLGVYFCSQSTHVPWTFGGGTKLEIK

SEQ ID NO: 27 - protein, 121 aa, Synthetic Construct
QVQLQQSGAELARPGASVKLSCKTSGYIFTNFGITWVKQRTGQGLEWIGENYPRRINTYYNEKFKGKATLTADKSSNTAYLELRSLTSEDSAVYFCSRKDIFGLSYALDYWGQGTSVTVSS

SEQ ID NO: 28 - protein, 107 aa, Synthetic Construct
DIVMTQSQKFMSTSVGDRVSVTCKASQNVGTNVAWYQHKPGQSPKALIYSASYQYSGVPDRFTGSGSGTDFTLTISNVQSEDLAEYICQQYKNYPYTFGGGTKLEIK

SEQ ID NO: 29 - protein, 5 aa, Synthetic Construct
NYGVS

SEQ ID NO: 30 - protein, 16 aa, Synthetic Construct
VIWGDGSTNYHSALIS

SEQ ID NO: 31 - protein, 14 aa, Synthetic Construct
PASYYGRRTYAMDF

SEQ ID NO: 32 - protein, 8 aa, Synthetic Construct
GFSLTNYG

SEQ ID NO: 33 - protein, 7 aa, Synthetic Construct
IWGDGST

SEQ ID NO: 34 - protein, 16 aa, Synthetic Construct
AKPASYYGRRTYAMDF

SEQ ID NO: 35 - protein, 10 aa, Synthetic Construct
RASSSVSYMH

SEQ ID NO: 36 - protein, 7 aa, Synthetic Construct
ATSHLAS

SEQ ID NO: 37 - protein, 10 aa, Synthetic Construct
QQWSSNPPMT

SEQ ID NO: 38 - protein, 5 aa, Synthetic Construct
SSVSY

SEQ ID NO: 39 - skipped

SEQ ID NO: 40 - protein, 5 aa, Synthetic Construct
SYWIT

SEQ ID NO: 41 - protein, 17 aa, Synthetic Construct
DFYPRNGDTNYNKKFKN

SEQ ID NO: 42 - protein, 12 aa, Synthetic Construct
SRAYYGRRGFDY

SEQ ID NO: 43 - protein, 8 aa, Synthetic Construct
GYTFSSYW

SEQ ID NO: 44 - protein, 8 aa, Synthetic Construct
FYPRNGDT

SEQ ID NO: 45 - protein, 14 aa, Synthetic Construct
ARSRAYYGRRGFDY

SEQ ID NO: 46 - protein, 10 aa, Synthetic Construct
SAGSSVSYMY

SEQ ID NO: 47 - protein, 7 aa, Synthetic Construct
DTSNLAS

SEQ ID NO: 48 - protein, 9 aa, Synthetic Construct
QQWSNYPLT

SEQ ID NO: 49 - protein, 5 aa, Synthetic Construct
SSVSY

SEQ ID NO: 50 - skipped

SEQ ID NO: 51 - protein, 5 aa, Synthetic Construct
SYNMN

SEQ ID NO: 52 - protein, 17 aa, Synthetic Construct
AIYPGNGDTSYNQKFKG

SEQ ID NO: 53 - protein, 9 aa, Synthetic Construct
VRLRYAMDY

SEQ ID NO: 54 - protein, 8 aa, Synthetic Construct
GYTFTSYN

SEQ ID NO: 55 - protein, 8 aa, Synthetic Construct
IYPGNGDT

SEQ ID NO: 56 - protein, 11 aa, Synthetic Construct
ARVRLRYAMDY

SEQ ID NO: 57 - protein, 11 aa, Synthetic Construct
KASQNVGTAVA

SEQ ID NO: 58 - protein, 7 aa, Synthetic Construct
SASNRYT

SEQ ID NO: 59 - protein, 9 aa, Synthetic Construct
QQYSSYPWT

SEQ ID NO: 60 - protein, 6 aa, Synthetic Construct
QNVGTA

SEQ ID NO: 61 - skipped

SEQ ID NO: 62 - protein, 5 aa, Synthetic Construct
RYAMS

SEQ ID NO: 63 - protein, 17 aa, Synthetic Construct
TISDGGSYTYYPDNVKG

SEQ ID NO: 64 - protein, 13 aa, Synthetic Construct
DRYYYGKGGYFDV

SEQ ID NO: 65 - protein, 8 aa, Synthetic Construct
RFTFSRYA

SEQ ID NO: 66 - protein, 8 aa, Synthetic Construct
ISDGGSYT

SEQ ID NO: 67 - protein, 15 aa, Synthetic Construct
ARDRYYYGKGGYFDV

SEQ ID NO: 68 - protein, 11 aa, Synthetic Construct
RASENIYRNLA

SEQ ID NO: 69 - protein, 7 aa, Synthetic Construct
AATNLAD

SEQ ID NO: 70 - protein, 9 aa, Synthetic Construct
QHFWGTPRT

SEQ ID NO: 71 - protein, 6 aa, Synthetic Construct
ENIYRN

SEQ ID NO: 72 - skipped

SEQ ID NO: 73 - protein, 5 aa, Synthetic Construct
SYGIS

SEQ ID NO: 74 - protein, 17 aa, Synthetic Construct
EIYPRSGNTYYNEKFKG

SEQ ID NO: 75 - protein, 12 aa, Synthetic Construct
GRAYGRNYPMDY

SEQ ID NO: 76 - protein, 8 aa, Synthetic Construct
GYTFTSYG

SEQ ID NO: 77 - protein, 8 aa, Synthetic Construct
IYPRSGNT

SEQ ID NO: 78 - protein, 14 aa, Synthetic Construct
ARGRAYGRNYPMDY

SEQ ID NO: 79 - protein, 11 aa, Synthetic Construct
RASQSIGTSIH

SEQ ID NO: 80 - protein, 7 aa, Synthetic Construct
YASESIS

SEQ ID NO: 81 - protein, 9 aa, Synthetic Construct
QQSNSWPYT

SEQ ID NO: 82 - protein, 6 aa, Synthetic Construct
QSIGTS

SEQ ID NO: 83 - skipped

SEQ ID NO: 84 - protein, 5 aa, Synthetic Construct
SYGVN

SEQ ID NO: 85 - protein, 16 aa, Synthetic Construct
VIWSGGNTDYNAAFRS

SEQ ID NO: 86 - protein, 12 aa, Synthetic Construct
GQLGRPYWYFDV

SEQ ID NO: 87 - protein, 8 aa, Synthetic Construct
GFSLTSYG

SEQ ID NO: 88 - protein, 7 aa, Synthetic Construct
IWSGGNT

SEQ ID NO: 89 - protein, 14 aa, Synthetic Construct
ARGQLGRPYWYFDV

SEQ ID NO: 90 - protein, 11 aa, Synthetic Construct
KASQDVRTAVA

SEQ ID NO: 91 - protein, 7 aa, Synthetic Construct
WASTRHT

SEQ ID NO: 92 - protein, 9 aa, Synthetic Construct
QQHYSTPLT

SEQ ID NO: 93 - protein, 6 aa, Synthetic Construct
QDVRTA

SEQ ID NO: 94 - skipped

SEQ ID NO: 95 - protein, 5 aa, Synthetic Construct
NYLIE

SEQ ID NO: 96 - protein, 17 aa, Synthetic Construct
MINPGRGNTNYNEKFKG

SEQ ID NO: 97 - protein, 4 aa, Synthetic Construct
NWDV

SEQ ID NO: 98 - protein, 8 aa, Synthetic Construct
GYAFTNYL

SEQ ID NO: 99 - protein, 8 aa, Synthetic Construct
INPGRGNT

SEQ ID NO: 100 - protein, 6 aa, Synthetic Construct
ARNWDV

SEQ ID NO: 101 - protein, 16 aa, Synthetic Construct
RSSQSLVYSNGNTYLH

SEQ ID NO: 102 - protein, 7 aa, Synthetic Construct
KVSNRFS

SEQ ID NO: 103 - protein, 9 aa, Synthetic Construct
SQSTHVPWT

SEQ ID NO: 104 - protein, 11 aa, Synthetic Construct
QSLVYSNGNTY

SEQ ID NO: 105 - skipped

SEQ ID NO: 106 - protein, 5 aa, Synthetic Construct
NFGIT

SEQ ID NO: 107 - protein, 17 aa, Synthetic Construct
ENYPRRINTYYNEKFKG

SEQ ID NO: 108 - protein, 12 aa, Synthetic Construct
KDIFGLSYALDY

SEQ ID NO: 109 - protein, 8 aa, Synthetic Construct
GYIFTNFG

SEQ ID NO: 110 - protein, 8 aa, Synthetic Construct
NYPRRINT

SEQ ID NO: 111 - protein, 14 aa, Synthetic Construct
SRKDIFGLSYALDY

SEQ ID NO: 112 - protein, 11 aa, Synthetic Construct
KASQNVGTNVA

SEQ ID NO: 113 - protein, 7 aa, Synthetic Construct
SASYQYS

SEQ ID NO: 114 - protein, 9 aa, Synthetic Construct
QQYKNYPYT

SEQ ID NO: 115 - protein, 6 aa, Synthetic Construct
QNVGTN

SEQ ID NO: 116 - skipped

SEQ ID NO: 117 - protein, 15 aa, Synthetic Construct
GGGGSGGGGSGGGGS

SEQ ID NO: 118 - protein, 107 aa, Synthetic Construct
DIQLTQSPSFLSASVGDRVTITCRASSSVSYMHWYQQKPGKAPKPLIYATSHLASGVPSRFSGSGSGTEFTLTISSLQPEDFATYYCQQWSSNPPMTFGGGTKVEIK

SEQ ID NO: 119 - protein, 107 aa, Synthetic Construct
DIQLTQSPSFLSASVGDRVTITCRASSSVSYMHWYQQKPGKAPKPWIYATSHLASGVPSRFSGSGSGTEFTLTISSLQPEDFATYYCQQWSSNPPMTFGGGTKVEIK

SEQ ID NO: 120 - protein, 107 aa, Synthetic Construct
DIQLTQSPSFLSASVGDRVTITCRASSSVSYMHWYQQKPGKSPKPWIYATSHLASGVPSRFSGSGSGTEFTLTISSLQPEDFATYYCQQWSSNPPMTFGGGTKVEIK

SEQ ID NO: 121 - protein, 122 aa, Synthetic Construct
EVTLKESGPVLVKPTETLTLTCTVSGFSLSNYGVSWIRQPPGKALEWLAVIWGDGSTNYHSALISRLTISKDTSKSQVVLTMTNMDPVDTATYYCAKPASYYGRRTYAMDFWGQGTTVTVSS

SEQ ID NO: 122 - protein, 122 aa, Synthetic Construct
EVTLKESGPVLVKPTETLTLTCTVSGFSLTNYGVSWIRQPPGKALEWLAVIWGDGSTNYHSALISRLTISKDNSKSQVVLTMTNMDPVDTATYYCAKPASYYGRRTYAMDFWGQGTTVTVSS

SEQ ID NO: 123 - protein, 122 aa, Synthetic Construct
EVTLKESGPVLVKPTETLTLTCTVSGFSLTNYGVSWIRQPPGKALEWLAVIWGDGSTNYHSALISRLTIRKDNSKSQVVLTMTNMDPVDTATYYCAKPASYYGRRTYAMDFWGQGTTVTVSS

SEQ ID NO: 124 - protein, 122 aa, Synthetic Construct
EVTLKESGPVLVKPTETLTLTCTVSGFSLTNYGVSWIRQPPGKALEWLAVIWGDGSTNYHSALISRLTISKDNSKSQVFLTMTNMDPVDTATYYCAKPASYYGRRTYAMDFWGQGTTVTVSS

SEQ ID NO: 125 - protein, 122 aa, Synthetic Construct
EVTLKESGPVLVKPTETLTLTCTVSGFSLTNYGVSWIRQPPGKALEWLAVIWGDGSTNYHSALISRLTISKDNSKSQVVLTMTNMDPVDTATYYCAKPASYYGRRTYAMDFWGHGTTVTVSS

SEQ ID NO: 126 - protein, 95 aa, Synthetic Construct
DIQLTQSPSFLSASVGDRVTITCRASQGISSYLAWYQQKPGKAPKLLIYAASTLQSGVPSRFSGSGSGTEFTLTISSLQPEDFATYYCQQLNSYP

SEQ ID NO: 127 - protein, 10 aa, Synthetic Construct
FGGGTKVEIK

SEQ ID NO: 128 - protein, 100 aa, Synthetic Construct
QVTLKESGPVLVKPTETLTLTCTVSGFSLSNARMGVSWIRQPPGKALEWLAHIFSNDEKSYSTSLKSRLTISKDTSKSQVVLTMTNMDPVDTATYYCARI

SEQ ID NO: 129 - protein, 11 aa, Synthetic Construct
WGQGTTVTVSS

SEQ ID NO: 130 - protein, 106 aa, Synthetic Construct
EIVLTQSPATLSLSPGERATLSCSAGSSVSYMYWYQQKPGQAPRVLIYDTSNLASGIPARFSGSGSGTDFTLTISRLEPEDFAVYYCQQWSNYPLTFGQGTKLEIK

SEQ ID NO: 131 - protein, 106 aa, Synthetic Construct
EIVLTQSPATLSLSPGERATLSCSAGSSVSYMYWYQQKPGQSPRVLIYDTSNLASGIPARFSGSGSGTDFTLTISRLEPEDFAVYYCQQWSNYPLTFGQGTKLEIK

SEQ ID NO: 132 - protein, 121 aa, Synthetic Construct
EVQLVQSGAEVKKPGASVKVSCKASGYTFSSYWITWVRQAPGQGLEWMGDFYPRNGDTNYNKKFKNRVTMTVDTSTSTVYMELSSLRSEDTAVYYCARSRAYYGRRGFDYWGQGTTVTVSS

SEQ ID NO: 133 - protein, 121 aa, Synthetic Construct
EVQLVQSGAEVKKPGASVKVSCKASGYTFSSYWITWVRQAPGQGLEWMGDFYPRNGDTNYNKKFKNRVTMTVDTSTSTAYMELSSLRSEDTAVYYCARSRAYYGRRGFDYWGQGTTVTVSS

SEQ ID NO: 134 - protein, 121 aa, Synthetic Construct
EVQLVQSGAEVKKPGASVKVSCKASGYTFSSYWITWVRQAPGQGLEWMGDFYPRSGDTNYNKKFKNRVTMTVDTSTSTAYMELSSLRSEDTAVYYCARSRAYYGRRGFDYWGQGTTVTVSS

SEQ ID NO: 135 - protein, 121 aa, Synthetic Construct
EVQLVQSGAEVKKPGASVKVSCKASGYTFSSYWITWVRQAPGQGLEWMGDFYPRNGDTNYNKKFKNRVTLTVDTSTSTAYMELSSLRSEDTAVYYCARSRAYYGRRGFDYWGQGTTVTVSS

SEQ ID NO: 136 - protein, 121 aa, Synthetic Construct
EVQLVQSGAEVKKPGASVKVSCKASGYTFSSYWITWVRQAPGQGLEWMGDFYPRNADTNYNKKFKNRVTLTVDTSTSTAYMELSSLRSEDTAVYYCARSRAYYGRRGFDYWGQGTTVTVSS

SEQ ID NO: 137 - protein, 121 aa, Synthetic Construct
EVQLQQSGAEVKKPGASVKVSCKASGYTFSSYWITWVRQAPGQGLEWMGDFYPRNGDTNYNKKFKNRVTMTVDTSTSTAYMELSSLRSEDTAVYYCARSRAYYGRRGFDYWGQGTTVTVSS

SEQ ID NO: 138 - protein, 90 aa, Synthetic Construct
EIVLTQSPATLSLSPGERATLSCRASQSVSSSYLAWYQQKPGQAPRLLIYGASSRATGIPARFSGSGSGTDFTLTISRLEPEDFAVYYCQ

SEQ ID NO: 139 - protein, 10 aa, Synthetic Construct
FGQGTKLEIK

SEQ ID NO: 140 - protein, 98 aa, Synthetic Construct
QVQLVQSGAEVKKPGASVKVSCKASGYTFTSYYMHWVRQAPGQGLEWMGIINPSGGSTSYAQKFQGRVTMTRDTSTSTVYMELSSLRSEDTAVYYCAR

SEQ ID NO: 141 - protein, 11 aa, Synthetic Construct
WGQGTTVTVSS

SEQ ID NO: 142 - protein, 17 aa, Synthetic Construct
DFYPRSGDTNYNKKFKN

SEQ ID NO: 143 - protein, 17 aa, Synthetic Construct
DFYPRNADTNYNKKFKN

SEQ ID NO: 144 - protein, 107 aa, Synthetic Construct
DIQMTQSPSSLSASVGDRVTITCKASQNVGTAVAWYQQKPGKSPKLLISSASNRYTGVPSRFSGSGSGTDFTLTISSLQPEDFATYYCQQYSSYPWTFGGGTKVEIK

SEQ ID NO: 145 - protein, 107 aa, Synthetic Construct
DIVMTQSPDSLAVSLGERATINCKASQNVGTAVAWYQQKPGQSPKLLISSASNRYTGVPDRFSGSGSGTDFTLTISSLQAEDVAVYYCQQYSSYPWTFGGGTKVEIK

SEQ ID NO: 146 - protein, 118 aa, Synthetic Construct
EVQLVQSGAEVKKPGASVKVSCKASGYTFTSYNMNWVRQAPGQRLEWMGAIYPGNGDTSYNQKFKGRVTITVDKSASTAYMELSSLRSEDTAVYYCARVRLRYAMDYWGQGTTVTVSS

SEQ ID NO: 147 - protein, 118 aa, Synthetic Construct
EAQLVQSGAEVKKPGASVKVSCKASGYTFTSYNMNWVRQAPGQRLEWMGAIYPGNGDTSYNQKFKGRVTITVDKSASTAYMELSSLRSEDTAVYYCARVRLRYAMDYWGQGTTVTVSS

SEQ ID NO: 148 - protein, 118 aa, Synthetic Construct
EAQLVQSGAEVKKPGASVKVSCKASGYTFTSYNMNWVRQAPGQRLEWMGAIYPGSGDTSYNQKFKGRVTITVDKSASTAYMELSSLRSEDTAVYYCARVRLRYAMDYWGQGTTVTVSS

SEQ ID NO: 149 - protein, 118 aa, Synthetic Construct
EAQLVQSGAEVKKPGASVKVSCKASGYTFTSYNMNWVRQAPGQRLEWMGAIYPGNGDTSYNQKFKGRVTLTVDKSASTAYMELSSLRSEDTAVYYCARVRLRYAMDYWGQGTTVTVSS

SEQ ID NO: 150 - protein, 118 aa, Synthetic Construct
EAYLQQSGAEVKKPGASVKVSCKASGYTFTSYNMNWVRQAPGQRLEWMGAIYPGNGDTSYNQKFKGRVTITVDKSASTAYMELSSLRSEDTAVYYCARVRLRYAMDYWGQGTTVTVSS

SEQ ID NO: 151 - protein, 118 aa, Synthetic Construct
EAYLQQSGAEVKKPGASVKVSCKASGYTFTSYNMNWVRQAPGQRLEWMGAIYPGNADTSYNQKFKGRVTITVDKSASTAYMELSSLRSEDTAVYYCARVRLRYAMDYWGQGTTVTVSS

SEQ ID NO: 152 - protein, 118 aa, Synthetic Construct
EAQLVQSGAEVKKPGASVKVSCKASGYTFTSYNMNWVRQAPRQGLEWMGAIYPGNGDTSYNQKFKGRVTITVDKSASTAYMELSSLRSEDTAVYYCARVRLRYAMDYWGQGTTVTVSS

SEQ ID NO: 153 - protein, 101 aa, Synthetic Construct
DIVMTQSPDSLAVSLGERATINCKSSQSVLYSSNNKNYLAWYQQKPGQPPKLLIYWASTRESGVPDRFSGSGSGTDFTLTISSLQAEDVAVYYCQQYYSTP

SEQ ID NO: 154 - protein, 95 aa, Synthetic Construct
DIQMTQSPSSLSASVGDRVTITCRASQSISSYLNWYQQKPGKAPKLLIYAASSLQSGVPSRFSGSGSGTDFTLTISSLQPEDFATYYCQQSYSTP

SEQ ID NO: 155 - protein, 10 aa, Synthetic Construct
FGGGTKVEIK

SEQ ID NO: 156 - protein, 98 aa, Synthetic Construct
QVQLVQSGAEVKKPGASVKVSCKASGYTFTSYAMHWVRQAPGQRLEWMGWINAGNGNTKYSQKFQGRVTITRDTSASTAYMELSSLRSEDTAVYYCAR

SEQ ID NO: 157 - protein, 11 aa, Synthetic Construct
WGQGTTVTVSS

SEQ ID NO: 158 - protein, 17 aa, Synthetic Construct
AIYPGSGDTSYNQKFKG

SEQ ID NO: 159 - protein, 17 aa, Synthetic Construct
AIYPGNADTSYNQKFKG

SEQ ID NO: 160 - protein, 107 aa, Synthetic Construct
DIQMTQSPSSLSASVGDRVTITCRASENIYRNLAWYQQKPGKSPKLLVYAATNLADGVPSRFSGSGSGTDFTLTISSLQPEDFATYYCQHFWGTPRTFGGGTKVEIK

SEQ ID NO: 161 - protein, 107 aa, Synthetic Construct
DIQMTQSPSSLSASVGDRVTITCRASENIYRNLAWYQQKPGKSPQLLVYAATNLADGVPSRFSGSGSGTDFTLTISSLQPEDFATYYCQHFWGTPRTFGGGTKVEIK

SEQ ID NO: 162 - protein, 107 aa, Synthetic Construct
DIVMTQSPLSLPVTPGEPASISCRASENIYRNLAWYLQKPGQSPQLLVYAATNLADGVPDRFSGSGSGTDFTLKISRVEAEDVGVYYCQHFWGTPRTFGGGTKVEIK

SEQ ID NO: 163 - protein, 107 aa, Synthetic Construct
DIVMTQSPLSLPVTPGEPASISCRASENIYRNLAWYLQKQGQSPQLLVYAATNLADGVPDRFSGSGSGTDFTLKISRVEAEDVGVYYCQHFWGTPRTFGGGTKVEIK

SEQ ID NO: 164 - protein, 122 aa, Synthetic Construct
EVQLVESGGGLVQPGGSLRLSCAASGFTFSRYAMSWVRQAPGKGLEWVATISDGGSYTYYPDNVKGRFTISRDNAKNSLYLQMNSLRAEDTAVYYCARDRYYYGKGGYFDVWGQGTTVTVSS

SEQ ID NO: 165 - protein, 122 aa, Synthetic Construct
EVQLVESGGGLVQPGGSLRLSCAASRFTFSRYAMSWVRQAPGKGLEWVATISDGGSYTYYPDNVKGRFTISRDNAKNSLYLQMNSLRAEDTAVYYCARDRYYYGKGGYFDVWGQGTTVTVSS

SEQ ID NO: 166 - protein, 122 aa, Synthetic Construct
EVQLVESGGGLVQPGGSLRLSCAASRFTFSRYAMSWVRQAPEKRLEWVATISDGGSYTYYPDNVKGRFTISRDNAKNSLYLQMNSLRAEDTAVYYCARDRYYYGKGGYFDVWGQGTTVTVSS

SEQ ID NO: 167 - protein, 95 aa, Synthetic Construct; identical to SEQ ID NO: 154

SEQ ID NO: 168 - protein, 100 aa, Synthetic Construct
DIVMTQSPLSLPVTPGEPASISCRSSQSLLHSNGYNYLDWYLQKPGQSPQLLIYLGSNRASGVPDRFSGSGSGTDFTLKISRVEAEDVGVYYCMQALQTP

SEQ ID NO: 169 - protein, 10 aa, Synthetic Construct
FGGGTKVEIK

SEQ ID NO: 170 - protein, 98 aa, Synthetic Construct
EVQLVESGGGLVQPGGSLRLSCAASGFTFSSYWMSWVRQAPGKGLEWVANIKQDGSEKYYVDSVKGRFTISRDNAKNSLYLQMNSLRAEDTAVYYCAR

SEQ ID NO: 171 - protein, 11 aa, Synthetic Construct
WGQGTTVTVSS

SEQ ID NO: 172 - protein, 107 aa, Synthetic Construct
EIVLTQSPDFQSVTPKEKVTITCRASQSIGTSIHWYQQKPDQSPKLLIKYASESISGIPSRFSGSGSGTDFTLTINSLEAEDAATYYCQQSNSWPYTFGGGTKVEIK

SEQ ID NO: 173 - protein, 107 aa, Synthetic Construct
EIVLTQSPDFQSVTPKEKVTITCRASQSIGTSIHWYQQKPDGSPKLLIKYASESISGIPSRFSGSGSGTDFTLTINSLEAEDAATYYCQQSNSWPYTFGGGTKVEIK

SEQ ID NO: 174 - protein, 107 aa, Synthetic Construct
EIVLTQSPDFQSVTPKEKVTITCRASQSIGTSIHWYQQKTDGSPKLLIKYASESISGIPSRFSGSGSGTDFTLTINSLEAEDAATYYCQQSNSWPYTFGGGTKVEIK

SEQ ID NO: 175 - protein, 107 aa, Synthetic Construct
EIVLTQSPATLSLSPGERATLSCRASQSIGTSIHWYQQKPGQSPRLLIKYASESISGIPARFSGSGSGTDFTLTISSLEPEDFAVYYCQQSNSWPYTFGGGTKVEIK

SEQ ID NO: 176 - protein, 121 aa, Synthetic Construct
EVQLVQSGAEVKKPGSSVKVSCKASGYTFSSYGISWVRQAPGQGLEWMGEIYPRSGNTYYNEKFKGRVTITADKSTSTAYMELSSLRSEDTAVYYCARGRAYGRNYPMDYWGQGTTVTVSS

SEQ ID NO: 177 - protein, 121 aa, Synthetic Construct
EVQLVQSGAEVKKPGSSVKVSCKASGYTFTSYGISWVRQAPGQGLEWMGEIYPRSGNTYYNEKFKGRVTITADKSTSTAYMELSSLRSEDTAVYYCARGRAYGRNYPMDYWGQGTTVTVSS

SEQ ID NO: 178 - protein, 121 aa, Synthetic Construct
EVQLVQSGAEVKKPGSSVKVSCKASGYTFTSYGISWVRQAPGQGLEWMGEIYPRSGNTYYNEKFKGRVTLTADKSTSTAYMELSSLRSEDTAVYYCARGRAYGRNYPMDYWGQGTTVTVSS

SEQ ID NO: 179 - protein, 95 aa, Synthetic Construct
EIVLTQSPDFQSVTPKEKVTITCRASQSIGSSLHWYQQKPDQSPKLLIKYASQSFSGVPSRFSGSGSGTDFTLTINSLEAEDAATYYCHQSSSLP

SEQ ID NO: 180 - protein, 95 aa, Synthetic Construct
EIVLTQSPATLSLSPGERATLSCRASQSVSSYLAWYQQKPGQAPRLLIYDASNRATGIPARFSGSGSGTDFTLTISSLEPEDFAVYYCQQRSNWP

SEQ ID NO: 181 - protein, 10 aa, Synthetic Construct
FGGGTKVEIK

SEQ ID NO: 182 - protein, 98 aa, Synthetic Construct
QVQLVQSGAEVKKPGSSVKVSCKASGGTFSSYTISWVRQAPGQGLEWMGRIIPILGIANYAQKFQGRVTITADKSTSTAYMELSSLRSEDTAVYYCAR

SEQ ID NO: 183 - protein, 11 aa, Synthetic Construct
WGQGTTVTVSS

SEQ ID NO: 184 - protein, 107 aa, Synthetic Construct
DIVMTQSPDSLAVSLGERATINCKASQDVRTAVAWYQQKPGQSPKLLIYWASTRHTGVPDRFSGSGSGTDFTLTISSLQAEDVAVYYCQQHYSTPLTFGQGTKLEIK

SEQ ID NO: 185 - protein, 107 aa, Synthetic Construct
DIVMTQSPDSLAVSLGERATINCKASQDVRTAVAWYQQKPGQSPKLLIYWASTRHTGVPDRFSGSRSGTDFTLTISSLQAEDVAVYYCQQHYSTPLTFGQGTKLEIK

SEQ ID NO: 186 - protein, 107 aa, Synthetic Construct
DIVMTQSPDSLAVSLGERATINCKASQDVRTAVAWYQQKPGQSPKLLIYWASTRHTGVPDRFSGSRSGTDFTLTISSLQAEDVAVYYCQQHYSTPLTFGAGTKLEIK

SEQ ID NO: 187 - protein, 107 aa, Synthetic Construct
DIQMTQSPSSLSASVGDRVTITCKASQDVRTAVAWYQQKPGKSPKLLIYWASTRHTGVPDRFSGSGSGTDFTLTISSLQPEDVATYYCQQHYSTPLTFGQGTKLEIK

SEQ ID NO: 188 - protein, 120 aa, Synthetic Construct
EVTLKESGPVLVKPTETLTLTCTVSGFSLTSYGVNWIRQPPGKALEWLAVIWSGGNTDYNAAFRSRLTISKDNSKSQVVLTMTNMDPVDTATYYCARGQLGRPYWYFDVWGQGTTVTVSS

SEQ ID NO: 189 - protein, 120 aa, Synthetic Construct
EVTLKESGPVLVKPTETLTLTCTVSGFSLTSYGVNWIRQPPGKALEWLAVIWSGGNTDYNAAFRSRLTISKDNSKSQVFLTMTNMDPVDTATYYCARGQLGRPYWYFDVWGQGTTVTVSS

SEQ ID NO: 190 - protein, 120 aa, Synthetic Construct
EVTLKESGPVLVKPTETLTLTCTVSGFSLTSYGVNWIRQPPGKALEWLAVIWSGGNTDYNAAFRSRLTISKDNSKSQVFFTMTNMDPVDTATYYCARGQLGRPYWYFDVWGQGTTVTVSS

SEQ ID NO: 191 - protein, 101 aa, Synthetic Construct; identical to SEQ ID NO: 153

SEQ ID NO: 192 - protein, 95 aa, Synthetic Construct
DIQMTQSPSSLSASVGDRVTITCRASQGISNYLAWYQQKPGKVPKLLIYAASTLQSGVPSRFSGSGSGTDFTLTISSLQPEDVATYYCQKYNSAP

SEQ ID NO: 193 - protein, 10 aa, Synthetic Construct
FGQGTKLEIK

SEQ ID NO: 194 - protein, 100 aa, Synthetic Construct; identical to SEQ ID NO: 128

SEQ ID NO: 195 - protein, 11 aa, Synthetic Construct
WGQGTTVTVSS

SEQ ID NO: 196 - protein, 107 aa, Synthetic Construct; identical to SEQ ID NO: 187

SEQ ID NO: 197 - protein, 107 aa, Synthetic Construct
DIVMTQSPSSLSASVGDRVTITCKASQDVRTAVAWYQQKPGKSPKLLIYWASTRHTGVPDRFSGSGSGTDFTLTISSLQPEDVATYYCQQHYSTPLTFGQGTKLEIK

SEQ ID NO: 198 - protein, 120 aa, Synthetic Construct
QVQLKESGPVLVKPTETLTLTCTVSGFSLTSYGVNWIRQPPGKALEWLAVIWSGGNTDYNAAFRSRLTISKDNSKSQVVLTMTNMDPVDTATYYCARGQLGRPYWYFDVWGQGTTVTVSS

SEQ ID NO: 199 - protein, 120 aa, Synthetic Construct
QVQLKESGPVLVKPTETLTLTCTVSGFSLTSYGVNWIRQPPGKALEWLAVIWSGGNTDYNAAFRSRLTISKDNSKSQVVLTMTNMDPVDTATYYCARGQLGRPYWYFDVWGTGTTVTVSS

SEQ ID NO: 200 - protein, 120 aa, Synthetic Construct
EVTLKESGPVLVKPTETLTLTCTVSGFSLTSYGVNWIRQPPGKALEWLAVIWSGGNTDYNAAFRSRLSISKDNSKSQVVLTMTNMDPVDTATYYCARGQLGRPYWYFDVWGQGTTVTVSS

SEQ ID NO: 201 - protein, 120 aa, Synthetic Construct
EVTLKESGPVLVKPTETLTLTCTVSGFSLTSYGVNWIRQPPGKALEWLAVIWSGGNTDYNAAFRSRLTISKDNSKSQVVLKMTNMDPVDTATYYCARGQLGRPYWYFDVWGQGTTVTVSS

SEQ ID NO: 202 - protein, 95 aa, Synthetic Construct; identical to SEQ ID NO: 192

SEQ ID NO: 203 - protein, 10 aa, Synthetic Construct
FGQGTKLEIK

SEQ ID NO: 204 - protein, 100 aa, Synthetic Construct; identical to SEQ ID NO: 128

SEQ ID NO: 205 - protein, 11 aa, Synthetic Construct
WGQGTTVTVSS

SEQ ID NO: 206 - protein, 112 aa, Synthetic Construct
DIVMTQTPLSLPVTPGEPASISCRSSQSLVYSNGNTYLHWYLQKPGQSPQLLIYKVSNRFSGVPDRFSGSGSGTDFTLKISRVEAEDVGVYYCSQSTHVPWTFGGGTKVEIK

SEQ ID NO: 207 - protein, 112 aa, Synthetic Construct
DIVMTQTPLSLPVTPGEPASISCRSSQSLVYSNGNTYLHWYLQKPGQSPKLLIYKVSNRFSGVPDRFSGSGSGTDFTLKISRVEAEDVGVYYCSQSTHVPWTFGGGTKVEIK

SEQ ID NO: 208 - protein, 112 aa, Synthetic Construct
DIVMTQTPLSLPVTPGEPASISCRSSQSLVYSNANTYLHWYLQKPGQSPKLLIYKVSNRFSGVPDRFSGSGSGTDFTLKISRVEAEDVGVYYCSQSTHVPWTFGGGTKVEIK

SEQ ID NO: 209 - protein, 113 aa, Synthetic Construct
EVQLVQSGAEVKKPGSSVKVSCKASGYAFTNYLIEWVRQAPGQGLEWMGMINPGRGNTNYNEKFKGRVTITADKSTSTAYMELSSLRSEDTAVYYCARNWDVWGQGTTVTVSS

SEQ ID NO: 210 - protein, 113 aa, Synthetic Construct
EVQLVQSGAEVKKPGSSVKVSCKASGYAFTNYLIEWVRQAPGQGLEWMGMINPGRGNTNYNEKFKGRVTLTADKSTSTAYMELSSLRSEDTAVYYCARNWDVWGQGTTVTVSS

SEQ ID NO: 211 - protein, 113 aa, Synthetic Construct
EVQLVQSGAEVKKPGSSVKVSCKASGYAFTNYLIEWVRQAPGQGLEWMGMINPGRGNTNYNEKFKGRVTLTADKATSTAYMELSSLRSEDTAVYYCARNWDVWGQGTTVTVSS

SEQ ID NO: 212 - protein, 113 aa, Synthetic Construct
QVQLQQSGAEVKKPGSSVKVSCKASGYAFTNYLIEWVRQAPGQGLEWMGMINPGRGNTNYNEKFKGRVTLTADKSTSTAYMELSSLRSEDTAVYYCARNWDVWGQGTTVTVSS

SEQ ID NO: 213 - protein, 101 aa, Synthetic Construct
DIVMTQTPLSLPVTPGEPASISCRSSQSLLDSDDGNTYLDWYLQKPGQSPQLLIYTLSYRASGVPDRFSGSGSGTDFTLKISRVEAEDVGVYYCMQRIEFP

SEQ ID NO: 214 - protein, 10 aa, Synthetic Construct
FGGGTKVEIK

SEQ ID NO: 215 - protein, 98 aa, Synthetic Construct; identical to SEQ ID NO: 182

SEQ ID NO: 216 - protein, 11 aa, Synthetic Construct
WGQGTTVTVSS

SEQ ID NO: 217 - protein, 16 aa, Synthetic Construct
RSSQSLVYSNANTYLH

SEQ ID NO: 218 - protein, 112 aa, Synthetic Construct
DIVMTQTPLSLPVTPGEPASISCRSSQSLVYSNANTYLHWYLQKPGQSPQLLIYKVSNRFSGVPDRFSGSGSGTDFTLKISRVEAEDVGVYYCSQSTHVPWTFGGGTKVEIK

SEQ ID NO: 219 - protein, 112 aa, Synthetic Construct
DIVMTQTPLSLPVTPGEPASISCRSSQSLVYSNSNTYLHWYLQKPGQSPQLLIYKVSNRFSGVPDRFSGSGSGTDFTLKISRVEAEDVGVYYCSQSTHVPWTFGGGTKVEIK

SEQ ID NO: 220 - protein, 112 aa, Synthetic Construct
DIVMTQTPLSLPVTPGEPASISCRSSQSLVYSDGNTYLHWYLQKPGQSPQLLIYKVSNRFSGVPDRFSGSGSGTDFTLKISRVEAEDVGVYYCSQSTHVPWTFGGGTKVEIK

SEQ ID NO: 221 - protein, 112 aa, Synthetic Construct
DIVMTQTPLSLPVTPGEPASISCRSSQSLVYSQGNTYLHWYLQKPGQSPQLLIYKVSNRFSGVPDRFSGSGSGTDFTLKISRVEAEDVGVYYCSQSTHVPWTFGGGTKVEIK

SEQ ID NO: 222 - protein, 113 aa, Synthetic Construct; identical to SEQ ID NO: 212

SEQ ID NO: 223 - protein, 101 aa, Synthetic Construct; identical to SEQ ID NO: 213

SEQ ID NO: 224 - protein, 10 aa, Synthetic Construct
FGGGTKVEIK

SEQ ID NO: 225 - protein, 98 aa, Synthetic Construct; identical to SEQ ID NO: 182

SEQ ID NO: 226 - protein, 11 aa, Synthetic Construct
WGQGTTVTVSS

SEQ ID NO: 227 - protein, 16 aa, Synthetic Construct
RSSQSLVYSNANTYLH

SEQ ID NO: 228 - protein, 16 aa, Synthetic Construct
RSSQSLVYSNSNTYLH

SEQ ID NO: 229 - protein, 16 aa, Synthetic Construct
RSSQSLVYSDGNTYLH

SEQ ID NO: 230 - protein, 16 aa, Synthetic Construct
RSSQSLVYSQGNTYLH

SEQ ID NO: 231 - protein, 107 aa, Synthetic Construct
DIVMTQTPLSLSVTPGQPASISCKASQNVGTNVAWYLQKPGQSPQALIYSASYQYSGVPDRFSGSGSGTDFTLKISRVEAEDVGVYYCQQYKNYPYTFGGGTKVEIK

SEQ ID NO: 232 - protein, 107 aa, Synthetic Construct
DIVMTQTPLSLSVTPGQPASISCKASQNVGTNVAWYLHKPGQSPQALIYSASYQYSGVPDRFSGSGSGTDFTLKISRVEAEDVGVYICQQYKNYPYTFGGGTKVEIK

SEQ ID NO: 233 - protein, 107 aa, Synthetic Construct
DIQMTQSPSSLSASVGDRVTITCKASQNVGTNVAWYQHKPGKSPKALIYSASYQYSGVPSRFSGSGSGTDFTLTISSLQPEDVATYICQQYKNYPYTFGGGTKVEIK

SEQ ID NO: 234 - protein, 121 aa, Synthetic Construct
EVQLVQSGAEVKKPGASVKVSCKASGYTFTNFGITWVRQAPGQRLEWMGENYPRRINTYYNEKFKGRVTITADKSASTAYMELSSLRSEDTAVYYCSRKDIFGLSYALDYWGQGTTVTVSS

SEQ ID NO: 235 - protein, 121 aa, Synthetic Construct
EVQLVQSGAEVKKPGASVKVSCKASGYIFTNFGITWVRQAPGQRLEWMGENYPRRINTYYNEKFKGRVTITADKSASTAYMELSSLRSEDTAVYYCSRKDIFGLSYALDYWGQGTTVTVSS

SEQ ID NO: 236 - protein, 121 aa, Synthetic Construct
EVQLVQSGAEVKKPGASVKVSCKTSGYIFTNFGITWVRQAPGQRLEWMGENYPRRINTYYNEKFKGRVTITADKSASTAYMELSSLRSEDTAVYYCSRKDIFGLSYALDYWGQGTTVTVSS

SEQ ID NO: 237 - protein, 121 aa, Synthetic Construct
EVQLVQSGAEVKKPGASVKVSCKTSGYIFTNFGITWVRQAPGQRLEWMGENYPRRINTYYNEKFKGRVTLTADKSASTAYMELSSLRSEDTAVYYCSRKDIFGLSYALDYWGQGTTVTVSS

SEQ ID NO: 238 - protein, 121 aa, Synthetic Construct
EVQLVQSGAEVKKPGASVKVSCKASGYIFTNFGITWVRQAPGQRLEWMGENYPRRINTYYNEKFKGRVTITADKSSNTAYMELSSLRSEDTAVYYCSRKDIFGLSYALDYWGQGTTVTVSS

SEQ ID NO: 239 - protein, 95 aa, Synthetic Construct; identical to SEQ ID NO: 192

SEQ ID NO: 240 - protein, 100 aa, Synthetic Construct
DIVMTQTPLSLSVTPGQPASISCKSSQSLLHSDGKTYLYWYLQKPGQSPQLLIYEVSSRFSGVPDRFSGSGSGTDFTLKISRVEAEDVGVYYCMQGIHLP

SEQ ID NO: 241 - protein, 10 aa, Synthetic Construct
FGGGTKVEIK

SEQ ID NO: 242 - protein, 98 aa, Synthetic Construct; identical to SEQ ID NO: 156

SEQ ID NO: 243 - protein, 11 aa, Synthetic Construct
WGQGTTVTVSS